European Patent Specification EP 4 010 329 B9, published October 4, 2023. Title: NOVEL COMPOUNDS. Applicant: Artios Pharma Limited. The sequence listing filed with the application follows.

SEQUENCE LISTING (2 sequences)

SEQ ID NO: 1 - DNA, 14 bp, Artificial
  Synthetic Primer
gcggctgtcataag

SEQ ID NO: 2 - DNA, 51 bp, Artificial
  Synthetic Primer
gctacattgacaatggcatcaaatctcagattgcgtcttatgacagccgcg